European Patent Application EP 4 253 550 A1, published October 4, 2023. Title: Method for the manufacture of a viral, a vector or any transport system and cancer-specific CRISPR complexes. Applicant: GenCC GmbH & Co. KG. The sequence listing filed with the application follows.

SEQUENCE LISTING (35 sequences)

SEQ ID NO: 1 - RNA, 36 nt, Synthetic sequence
gaagggugugaccgcaacguguuuuagagcuaugcu

SEQ ID NO: 2 - RNA, 36 nt, Synthetic sequence
guugccguagagcuugcccaguuuuagagcuaugcu

SEQ ID NO: 3 - RNA, 36 nt, Synthetic sequence
aacaccucggaggucuaccaguuuuagagcuaugcu

SEQ ID NO: 4 - RNA, 36 nt, Synthetic sequence
ccaaggagcucaggauguaaguuuuagagcuaugcu

SEQ ID NO: 5 - RNA, 36 nt, Synthetic sequence
aauucuuggcagguaaaggcguuuuagagcuaugcu

SEQ ID NO: 6 - RNA, 36 nt, Synthetic sequence
ggcagcgcuauaauaauaggguuuuagagcuaugcu

SEQ ID NO: 7 - RNA, 36 nt, Synthetic sequence
caacugcccacaggaucaucguuuuagagcuaugcu

SEQ ID NO: 8 - RNA, 36 nt, Synthetic sequence
caccgaggacaccugcgucaguuuuagagcuaugcu

SEQ ID NO: 9 - RNA, 36 nt, Synthetic sequence
ggccuucacagagacgaggcguuuuagagcuaugcu

SEQ ID NO: 10 - DNA, 3 bp, Homo sapiens
agg

SEQ ID NO: 11 - DNA, 3 bp, Homo sapiens
tgg

SEQ ID NO: 12 - DNA, 3 bp, Homo sapiens
ggg

SEQ ID NO: 13 - DNA, 3 bp, Homo sapiens
agg

SEQ ID NO: 14 - DNA, 3 bp, Homo sapiens
ggg

SEQ ID NO: 15 - DNA, 3 bp, Homo sapiens
cgg

SEQ ID NO: 16 - DNA, 3 bp, Homo sapiens
cgg

SEQ ID NO: 17 - DNA, 3 bp, Homo sapiens
cgg

SEQ ID NO: 18 - DNA, 20 bp, Synthetic sequence
gttcagcccttggagaatga

SEQ ID NO: 19 - DNA, 21 bp, Synthetic sequence
tgccagaggacagagagatta

SEQ ID NO: 20 - DNA, 20 bp, Synthetic sequence
gttcagcccttggagaatga

SEQ ID NO: 21 - DNA, 21 bp, Synthetic sequence
tgccagaggacagagagatta

SEQ ID NO: 22 - DNA, 20 bp, Synthetic sequence
gttcagcccttggagaatga

SEQ ID NO: 23 - DNA, 21 bp, Synthetic sequence
tgccagaggacagagagatta

SEQ ID NO: 24 - DNA, 20 bp, Synthetic sequence
gttcagcccttggagaatga

SEQ ID NO: 25 - DNA, 21 bp, Synthetic sequence
tgccagaggacagagagatta

SEQ ID NO: 26 - DNA, 20 bp, Synthetic sequence
gttcagcccttggagaatga

SEQ ID NO: 27 - DNA, 21 bp, Synthetic sequence
tgccagaggacagagagatta

SEQ ID NO: 28 - DNA, 20 bp, Synthetic sequence
gttcagcccttggagaatga

SEQ ID NO: 29 - DNA, 21 bp, Synthetic sequence
tgccagaggacagagagatta

SEQ ID NO: 30 - DNA, 20 bp, Synthetic sequence
gttcagcccttggagaatga

SEQ ID NO: 31 - DNA, 21 bp, Synthetic sequence
tgccagaggacagagagatta

SEQ ID NO: 32 - DNA, 20 bp, Synthetic sequence
gttcagcccttggagaatga

SEQ ID NO: 33 - DNA, 21 bp, Synthetic sequence
tgccagaggacagagagatta

SEQ ID NO: 34 - DNA, 20 bp, Synthetic sequence
gttcagcccttggagaatga

SEQ ID NO: 35 - DNA, 21 bp, Synthetic sequence
tgccagaggacagagagatta